European Patent Application EP 4 148 147 A1, published March 15, 2023. Title: MEANS AND METHOD FOR THE DIAGNOSIS AND TREATMENT OF AUTISM SPECTRUM DISORDERS BASED ON THE DETECTION AND MODULATION OF A DEUBIQUITINASE. Applicant: Universitätsmedizin der Johannes Gutenberg-Universität Mainz. The sequence listing filed with the application follows.

SEQUENCE LISTING (5 sequences)

SEQ ID NO: 1 - protein, 956 aa, Homo Sapiens
MSSGLWSQEKVTSPYWEERIFYLLLQECSVTDKQTQKLLKVPKGSIGQYIQDRSVGHSRIPSAKGKKNQIGLKILEQPHAVLFVDEKDVVEINEKFTELLLAITNCEERFSLFKNRNRLSKGLQIDVGCPVKVQLRSGEEKFPGVVRFRGPLLAERTVSGIFFGVELLEEGRGQGFTDGVYQGKQLFQCDEDCGVFVALDKLELIEDDDTALESDYAGPGDTMQVELPPLEINSRVSLKVGETIESGTVIFCDVLPGKESLGYFVGVDMDNPIGNWDGRFDGVQLCSFACVESTILLHINDIIPALSESVTQERRPPKLAFMSRGVGDKGSSSHNKPKATGSTSDPGNRNRSELFYTLNGSSVDSQPQSKSKNTWYIDEVAEDPAKSLTEISTDFDRSSPPLQPPPVNSLTTENRFHSLPFSLTKMPNTNGSIGHSPLSLSAQSVMEELNTAPVQESPPLAMPPGNSHGLEVGSLAEVKENPPFYGVIRWIGQPPGLNEVLAGLELEDECAGCTDGTFRGTRYFTCALKKALFVKLKSCRPDSRFASLQPVSNQIERCNSLAFGGYLSEVVEENTPPKMEKEGLEIMIGKKKGIQGHYNSCYLDSTLFCLFAFSSVLDTVLLRPKEKNDVEYYSETQELLRTEIVNPLRIYGYVCATKIMKLRKILEKVEAASGFTSEEKDPEEFLNILFHHILRVEPLLKIRSAGQKVQDCYFYQIFMEKNEKVGVPTIQQLLEWSFINSNLKFAEAPSCLIIQMPRFGKDFKLFKKIFPSLELNITDLLEDTPRQCRICGGLAMYECRECYDDPDISAGKIKQFCKTCNTQVHLHPKRLNHKYNPVSLPKDLPDWDWRHGCIPCQNMELFAVLCIETSHYVAFVKYGKDDSAWLFFDSMADRDGGQNGFNIPQVTPCPEVGEYLKMSLEDLHSLDSRRIQGCARRLLCDAYMCMYQSPTMSLYK

SEQ ID NO: 2 - protein, 953 aa, Homo Sapiens
MSSGLWSQEKVTSPYWEERIFYLLLQECSVTDKQTQKLLKVPKGSIGQYIQDRSVGHSRIPSAKGKKNQIGLKILEQPHAVLFVDEKDVVEINEKFTELLLAITNCEERFSLFKNRNRLSKGLQIDVGCPVKVQLRSGEEKFPGVVRFRGPLLAERTVSGIFFGVELLEEGRGQGFTDGVYQGKQLFQCDEDCGVFVALDKLELIEDDDTALESDYAGPGDTMQVELPPLEINSRVSLKVGETIESGTVIFCDVLPGKESLGYFVGVDMDNPIGNWDGRFDGVQLCSFACVESTILLHINDIIPESVTQERRPPKLAFMSRGVGDKGSSSHNKPKATGSTSDPGNRNRSELFYTLNGSSVDSQPQSKSKNTWYIDEVAEDPAKSLTEISTDFDRSSPPLQPPPVNSLTTENRFHSLPFSLTKMPNTNGSIGHSPLSLSAQSVMEELNTAPVQESPPLAMPPGNSHGLEVGSLAEVKENPPFYGVIRWIGQPPGLNEVLAGLELEDECAGCTDGTFRGTRYFTCALKKALFVKLKSCRPDSRFASLQPVSNQIERCNSLAFGGYLSEVVEENTPPKMEKEGLEIMIGKKKGIQGHYNSCYLDSTLFCLFAFSSVLDTVLLRPKEKNDVEYYSETQELLRTEIVNPLRIYGYVCATKIMKLRKILEKVEAASGFTSEEKDPEEFLNILFHHILRVEPLLKIRSAGQKVQDCYFYQIFMEKNEKVGVPTIQQLLEWSFINSNLKFAEAPSCLIIQMPRFGKDFKLFKKIFPSLELNITDLLEDTPRQCRICGGLAMYECRECYDDPDISAGKIKQFCKTCNTQVHLHPKRLNHKYNPVSLPKDLPDWDWRHGCIPCQNMELFAVLCIETSHYVAFVKYGKDDSAWLFFDSMADRDGGQNGFNIPQVTPCPEVGEYLKMSLEDLHSLDSRRIQGCARRLLCDAYMCMYQSPTMSLYK

SEQ ID NO: 3 - protein, 955 aa, Mus Musculus
MSSGLWSQEKVTSPYWEERIFYLLLQECSVTDKQTQKLLKVPKGSIGQYIQDRSVGHSRVPSTKGKKNQIGLKILEQPHAVLFVDEKDVVEINEKFTELLLAITNCEERLSLFRNRLRLSKGLQVDVGSPVKVQLRSGEEKFPGVVRFRGPLLAERTVSGIFFGVELLEEGRGQGFTDGVYQGKQLFQCDEDCGVFVALDKLELIEDDDNGLESDFAGPGDTMQVEPPPLEINSRVSLKVGESTESGTVIFCDVLPGKESLGYFVGVDMDNPIGNWDGRFDGVQLCSFASVESTILLHINDIIPALSDSVTQERRPPKLAFMSRGVGDKGSSSHNKPKVTGSTSDPGSRNRSELFYTLNGSSVDSQQSKSKNPWYIDEVAEDPAKSLTEMSSDFGHSSPPPQPPSMNSLSSENRFHSLPFSLTKMPNTNGSMAHSPLSLSVQSVMGELNSTPVQESPPLPISSGNAHGLEVGSLAEVKENPPFYGVIRWIGQPPGLSDVLAGLELEDECAGCTDGTFRGTRYFTCALKKALFVKLKSCRPDSRFASLQPVSNQIERCNSLAFGGYLSEVVEENTPPKMEKEGLEIMIGKKKGIQGHYNSCYLDSTLFCLFAFSSALDTVLLRPKEKNDIEYYSETQELLRTEIVNPLRIYGYVCATKIMKLRKILEKVEAASGFTSEEKDPEEFLNILFHDILRVEPLLKIRSAGQKVQDCNFYQIFMEKNEKVGVPTIQQLLEWSFINSNLKFAEAPSCLIIQMPRFGKDFKLFKKIFPSLELNITDLLEDTPRQCRICGGLAMYECRECYDDPDISAGKIKQFCKTCSTQVHLHPRRLNHSYHPVSLPKDLPDWDWRHGCIPCQKMELFAVLCIETSHYVAFVKYGKDDSAWLFFDSMADRDGGQNGFNIPQVTPCPEVGEYLKMSLEDLHSLDSRRIQGCARRLLCDAYMCMYQSPTMSLYK

SEQ ID NO: 4 - protein, 952 aa, Mus Musculus
MSSGLWSQEKVTSPYWEERIFYLLLQECSVTDKQTQKLLKVPKGSIGQYIQDRSVGHSRVPSTKGKKNQIGLKILEQPHAVLFVDEKDVVEINEKFTELLLAITNCEERLSLFRNRLRLSKGLQVDVGSPVKVQLRSGEEKFPGVVRFRGPLLAERTVSGIFFGVELLEEGRGQGFTDGVYQGKQLFQCDEDCGVFVALDKLELIEDDDNGLESDFAGPGDTMQVEPPPLEINSRVSLKVGESTESGTVIFCDVLPGKESLGYFVGVDMDNPIGNWDGRFDGVQLCSFASVESTILLHINDIIPDSVTQERRPPKLAFMSRGVGDKGSSSHNKPKVTGSTSDPGSRNRSELFYTLNGSSVDSQQSKSKNPWYIDEVAEDPAKSLTEMSSDFGHSSPPPQPPSMNSLSSENRFHSLPFSLTKMPNTNGSMAHSPLSLSVQSVMGELNSTPVQESPPLPISSGNAHGLEVGSLAEVKENPPFYGVIRWIGQPPGLSDVLAGLELEDECAGCTDGTFRGTRYFTCALKKALFVKLKSCRPDSRFASLQPVSNQIERCNSLAFGGYLSEVVEENTPPKMEKEGLEIMIGKKKGIQGHYNSCYLDSTLFCLFAFSSALDTVLLRPKEKNDIEYYSETQELLRTEIVNPLRIYGYVCATKIMKLRKILEKVEAASGFTSEEKDPEEFLNILFHDILRVEPLLKIRSAGQKVQDCNFYQIFMEKNEKVGVPTIQQLLEWSFINSNLKFAEAPSCLIIQMPRFGKDFKLFKKIFPSLELNITDLLEDTPRQCRICGGLAMYECRECYDDPDISAGKIKQFCKTCSTQVHLHPRRLNHSYHPVSLPKDLPDWDWRHGCIPCQKMELFAVLCIETSHYVAFVKYGKDDSAWLFFDSMADRDGGQNGFNIPQVTPCPEVGEYLKMSLEDLHSLDSRRIQGCARRLLCDAYMCMYQSPTMSLYK

SEQ ID NO: 5 - protein, 318 aa, Mus Musculus
MSSGLWSQEKVTSPYWEERIFYLLLQECSVTDKQTQKLLKVPKGSIGQYIQDRSVGHSRVPSTKGKKNQIGLKILEQPHAVLFVDEKDVVEINEKFTELLLAITNCEERLSLFRNRLRLSKGLQVDVGSPVKVQLRSGEEKFPGVVRFRGPLLAERTVSGIFFGVELLEEGRGQGFTDGVYQGKQLFQCDEDCGVFVALDKLELIEDDDNGLESDFAGPGDTMQVEPPPLEINSRVSLKVGESTESGTVIFCDVLPGKESLGYFVGVDMDNPIGNWDGRFDGVQLCSFASVESTILLHINDIIPGTSKNILDQQLKGK